European Patent Specification EP 3 244 920 B1, published June 7, 2023. Title: FOOT-AND-MOUTH DISEASE VACCINE. Applicant: Dominowski, Paul Joseph Hardham, John Morgan Jackson, James Alan Gay, Cyril Gerard Rodriguez, Luis Leandro Krug, Peter William Rieder, Aida Elizabeth. The sequence listing filed with the application follows.

SEQUENCE LISTING (30 sequences)

SEQ ID NO: 1 - DNA, 23 bp, Artificial Sequence
  CpG oligonucleotide
tcgtcgacgatcggcgcgcgccg

SEQ ID NO: 2 - DNA, 23 bp, Artificial Sequence
  CpG oligonucleotide
tcgacgtcgatcggcgcgcgccg

SEQ ID NO: 3 - DNA, 24 bp, Artificial Sequence
  CpG oligonucleotide
tcgacgtcgatcggcgcgcgccgt

SEQ ID NO: 4 - DNA, 23 bp, Artificial Sequence
  CpG oligonucleotide
  misc_feature (1)..(1): 5'-Iodo-2'-deoxyuridine
ncgacgtcgatcggcgcgcgccg

SEQ ID NO: 5 - DNA, 24 bp, Artificial Sequence
  CpG oligonucleotide
  misc_feature (1)..(1): 5'-Iodo-2'-deoxyuridine
ncgacgtcgatcggcgcgcgccgt

SEQ ID NO: 6 - DNA, 24 bp, Artificial Sequence
  CpG oligonucleotide
  misc_feature (1)..(1): 5'-Iodo-2'-deoxyuridine
ncgacgtcgatcggcgcgcgccgt

SEQ ID NO: 7 - DNA, 23 bp, Artificial Sequence
  CpG oligonucleotide
  misc_feature (1)..(1): 5'-Ethyl-2'-deoxyuridine
ncgacgtcgatcggcgcgcgccg

SEQ ID NO: 8 - DNA, 24 bp, Artificial Sequence
  CpG oligonucleotide
  misc_feature (1)..(1): 5'-Iodo-2'-deoxyuridine
ncgtcgacgatcggcggccgccgt

SEQ ID NO: 9 - DNA, 24 bp, Artificial Sequence
  CpG oligonucleotide
  misc_feature (1)..(1): 5'-Iodo-2'-deoxyuridine
ncgtcgacgatcggcggccgccgt

SEQ ID NO: 10 - DNA, 23 bp, Artificial Sequence
  CpG oligonucleotide
tcgtcgacgatcggcgcgcgccg

SEQ ID NO: 11 - DNA, 20 bp, Artificial Sequence
  RNA
uuguuguuguuguuguuguu

SEQ ID NO: 12 - DNA, 20 bp, Artificial Sequence
  RNA
uuauuauuauuauuauuauu

SEQ ID NO: 13 - DNA, 19 bp, Artificial Sequence
  RNA
aaacgcucagccaaagcag

SEQ ID NO: 14 - DNA, 21 bp, Artificial Sequence
  DNA/RNA
  misc_feature (11)..(17): ribonucleotides
tcgtcgttttguugugutttt

SEQ ID NO: 15 - DNA, 10867 bp, Artificial Sequence
  Fusion nucleotide:  Foot and Mouth Disease Virus (FMDV) and Bovine Rhinovirus Type 2 (BRV2)
ggggccggccaatccagtccggcgaccggctcgcagaaccaatctggcaacactggcagcataattaacaactactacatgcagcaataccagaactccatggacacacagttgggagacaatgccatcagtggaggctccaacgagggctccacggacacaacttcaacacacacaaccaacactcaaaacaatgactggttctcgaagctcgccagttcagcttttaccggtctgttcggtgcactgctcgccgacaagaagacagaggaaacgacacttcttgaggaccgcatcctcaccacccgcaacgggcacaccacctcgacgacccaatcgagtgtgggtgtcacacacgggtactccacagaggaggaccacgttgctgggcccaacacatcgggcctggagacgcgagtggtgcaggcagagagattctacaaaaagtacttgtttgactggacaacggacaaggcatttggacacctggaaaagctggagctcccgtccgaccaccacggtgtctttggacacttggtggactcgtacgcctatatgagaaatggctgggatgttgaggtgtccgctgttggcaaccagttcaacggcgggtgcctcctggtggccatggtacctgaatggaaggaatttgacacacgggagaaataccaactcacccttttcccgcaccagtttattagccccagaactaacatgactgcccacatcacggtcccctaccttggtgtgaacaggtatgatcagtacaagaagcataagccctggacattggttgtcatggtcgtgtcgccacttacggtcaacaacactagtgcggcacaaatcaaggtctacgccaacatagctccgacctatgttcacgtggccggtgaactcccctcgaaagaggggattttcccggttgcatgtgcggacggttacggaggattggtgacgacagacccgaagacagctgaccctgcttatggcaaggtgtacaacccgcctaggactaactaccctgggcgcttcaccaacctgttggacgtggccgaagcgtgtcccactttcctctgctttgacgacgggaaaccgtacgtcaccacgcggacggatgacacccgacttttggccaagtttgacctttcccttgccgcaaaacatatgtccaacacatacctgtcagggattgctcagtactacacacagtactctggcaccatcaatttgcatttcatgttcacaggttccactgattcaaaggcccgatacatggtggcctacatcccacctggggtggagacaccaccggacacacctgaaagggctgcccactgcattcacgctgaatgggacactggactaaactccaaattcactttctcaatcccgtacgtatccgccgcggattacgcgtacacagcgtctgacacggcagaaacaatcaacgtacagggatgggtctgcatctaccaaattacacacgggaaggctgaaaatgacaccttggtcgtgtcggttagcgccggcaaagactttgagttgcgcctcccgattgacccccgccagcagaccaccgctaccggggaatcagcagacccggtcaccaccaccgtggagaactacggcggtgagacacaaatccagagacgtcaccacacggacattggtttcatcatggacagatttgtgaagatccaaagcttgagcccaacacatgtcattgacctcatgcagactcaccaacacggtctggtgggtgccttgctgcgtgcagccacgtactacttttctgacctggaaattgttgtacggcacgaaggcaatctgacctgggtgcccaacggcgcccctgaatcagccctgttgaacaccagcaaccccactgcctacaacaaggcaccattcacgagactcgctctcccctacactgcgccgcaccgtgtgctggcaacagtgtacaacgggacgagtaagtatgctgtgggtggttcaggcagaagaggcgacatggggtctctcgcggcgcgagtcgtgaaacagcttcctgcttcatttaactacggtgcaatcaaggccgacgccatccacgaacttctcgtgcgcatgaaacgggccgagctctactgccccagaccgctgttggcaatagaggtgtcttcgcaagacaggcacaagcaaaagatcattgcaccagcaaagcagcttctgaattttgacctgcttaagctagccggagacgttgagtccaaccctgggcccttcttcttctccgacgttaggtcaaacttttccaagctggtagacacaatcaaccagatgcaggaagacatgtccacaaagcacggacctgactttaaccggttggtgtccgcttttgaggagttggccactggagtgaaagccatcaggaccggtcttgacgaggccaagccctggtacaagcttatcaagctcctgagccgcctgtcgtgcatggccgctgtggcagcacggtcaaaggacccagtccttgtggccatcatgctggctgacaccggtctcgagattctggacagcaccttcgtcgtgaagaagatctccgactcgctctccagtctcttccacgtgccggcccccgtcttcagtttcggagccccgattctgttagccgggttggtcaaggtcgcctcgagtttcttccggtccacgcccgaagaccttgagagagcagagaaacagctcaaagcacgtgacatcaacgacattttcgccattctcaagaacggcgagtggctggtcaaattgatccttgccatccgcgactggatcaaggcatggatagcctcagaagaaaagtttgtcaccacgacagacttggtacctagcatccttgaaaaacagcaggacctcaacgacccaagcaagtacaaggaagccaaggagtggctcgacaacgcgcgccaagcgtgtttgaagagcgggaacgtccacattgccaacctgtgcaaagtggtcgccccggcacccagcaggtcgagacccgagcccgtggtcgtttgcctccgtggcaagtccggtcagggcaagagtttccttgcaaacgtgctcgcacaagcaatctctacccatttcactggcaggaccgattcagtttggtactgcccgcctgaccctgaccacttcgacggttacaaccaacagactgtcgttgtgatggacgatttgggccagaaccccgacggcaaagacttcaagtacttcgcccaaatggtttcaacaacggggttcatcccgcccatggcatcgcttgaggataaaggcaaacccttcaacagtaaggtcatcatagcaaccaccaacctgtactcgggcttcaccccgaggactatggtgtgccctgatgccctgaaccggaggtttcactttgacatcgacgtgagcgccaaggacgggtacaaaattaacaacaaattggacatcatcaaagcacttgaagatactcacaccaacccagtggcaatgtttcagtacgactgtgcccttctcaacggcatggctgttgaaatgaagagaatgcaacaagatatgttcaagcctcaaccaccccttcagaacgtgtaccaactggttcaagaggtgattgagcgggtggagctccacgagaaggtgtcgagccacccgattttcaaacagatctcaattccttcccaaaaatccgtgttgtacttcctcattgagaaaggacagcacgaggcagcaattgaattctttgagggcatggtgcacgactccatcaaggaggagctccggccgctcatccaacaaacctcatttgtgaaacgcgcttttaagcgcctgaaggaaaactttgagattgttgccctatgtctgaccctcctggccaacatagtgatcatgatccgcgaaactcgcaagagacagaagatggtggacgatgcagtgagtgagtacattgagagagcaaacatcaccaccgacgacaagactcttgatgaggcggaaaagaaccctctggaaaccagcggtgccagcaccgtcggcttcagagagagacctctcccaggccaaaaggcgcgtaatgacgagaactccgagcccgcccagcctgctgaagagcaaccacaagctgaaggaccctacgctggcccgatggagagaccagttaaagttaaagtgaaagcaaaagccccggtcgttaaggaaggaccttacgagggaccggtgaagaagcctgttgctttgaaagtgaaagctaagaacttgatcgtcactgagagtggtgccccaccgaccgacttgcaaaagttggtcatgggcaacaccaagcccgttgagctcatccttgacgggaagacggtagccatttgctgtgctactggagttttcggcactgcttacctcgtgcctcgtcatcttttcgcagaaaagtacgacaagatcatgttggacggcagagccatgacagatagtgactacagagtgtttgagtttgagattaaagtaaaaggacaggacatgctctcagacgctgcgctcaggggccggccaatccagtccggcgaccggctcgcagaaccaatctggcaacactggcagcataattaacaactactacatgcagcaataccagaactccatggacacacagttgggagacaatgccatcagtggaggctccaacgagggctccacggacacaacttcaacacacacaaccaacactcaaaacaatgactggttctcgaagctcgccagttcagcttttaccggtctgttcggtgcactgctcgccgacaagaagacagaggaaacgacacttcttgaggaccgcatcctcaccacccgcaacgggcacaccacctcgacgacccaatcgagtgtgggtgtcacacacgggtactccacagaggaggaccacgttgctgggcccaacacatcgggcctggagacgcgagtggtgcaggcagagagattctacaaaaagtacttgtttgactggacaacggacaaggcatttggacacctggaaaagctggagctcccgtccgaccaccacggtgtctttggacacttggtggactcgtacgcctatatgagaaatggctgggatgttgaggtgtccgctgttggcaaccagttcaacggcgggtgcctcctggtggccatggtacctgaatggaaggaatttgacacacgggagaaataccaactcacccttttcccgcaccagtttattagccccagaactaacatgactgcccacatcacggtcccctaccttggtgtgaacaggtatgatcagtacaagaagcataagccctggacattggttgtcatggtcgtgtcgccacttacggtcaacaacactagtgcggcacaaatcaaggtctacgccaacatagctccgacctatgttcacgtggccggtgaactcccctcgaaagaggggattttcccggttgcatgtgcggacggttacggaggattggtgacgacagacccgaagacagctgaccctgcttatggcaaggtgtacaacccgcctaggactaactaccctgggcgcttcaccaacctgttggacgtggccgaagcgtgtcccactttcctctgctttgacgacgggaaaccgtacgtcaccacgcggacggatgacacccgacttttggccaagtttgacctttcccttgccgcaaaacatatgtccaacacatacctgtcagggattgctcagtactacacacagtactctggcaccatcaatttgcatttcatgttcacaggttccactgattcaaaggcccgatacatggtggcctacatcccacctggggtggagacaccaccggacacacctgaaagggctgcccactgcattcacgctgaatgggacactggactaaactccaaattcactttctcaatcccgtacgtatccgccgcggattacgcgtacacagcgtctgacacggcagaaacaatcaacgtacagggatgggtctgcatctaccaaattacacacgggaaggctgaaaatgacaccttggtcgtgtcggttagcgccggcaaagactttgagttgcgcctcccgattgacccccgccagcagaccaccgctaccggggaatcagcagacccggtcaccaccaccgtggagaactacggcggtgagacacaaatccagagacgtcaccacacggacattggtttcatcatggacagatttgtgaagatccaaagcttgagcccaacacatgtcattgacctcatgcagactcaccaacacggtctggtgggtgccttgctgcgtgcagccacgtactacttttctgacctggaaattgttgtacggcacgaaggcaatctgacctgggtgcccaacggcgcccctgaatcagccctgttgaacaccagcaaccccactgcctacaacaaggcaccattcacgagactcgctctcccctacactgcgccgcaccgtgtgctggcaacagtgtacaacgggacgagtaagtatgctgtgggtggttcaggcagaagaggcgacatggggtctctcgcggcgcgagtcgtgaaacagcttcctgcttcatttaactacggtgcaatcaaggccgacgccatccacgaacttctcgtgcgcatgaaacgggccgagctctactgccccagaccgctgttggcaatagaggtgtcttcgcaagacaggcacaagcaaaagatcattgcaccagcaaagcagcttctgaattttgacctgcttaagctagccggagacgttgagtccaaccctgggcccttcttcttctccgacgttaggtcaaacttttccaagctggtagacacaatcaaccagatgcaggaagacatgtccacaaagcacggacctgactttaaccggttggtgtccgcttttgaggagttggccactggagtgaaagccatcaggaccggtcttgacgaggccaagccctggtacaagcttatcaagctcctgagccgcctgtcgtgcatggccgctgtggcagcacggtcaaaggacccagtccttgtggccatcatgctggctgacaccggtctcgagattctggacagcaccttcgtcgtgaagaagatctccgactcgctctccagtctcttccacgtgccggcccccgtcttcagtttcggagccccgattctgttagccgggttggtcaaggtcgcctcgagtttcttccggtccacgcccgaagaccttgagagagcagagaaacagctcaaagcacgtgacatcaacgacattttcgccattctcaagaacggcgagtggctggtcaaattgatccttgccatccgcgactggatcaaggcatggatagcctcagaagaaaagtttgtcaccacgacagacttggtacctagcatccttgaaaaacagcaggacctcaacgacccaagcaagtacaaggaagccaaggagtggctcgacaacgcgcgccaagcgtgtttgaagagcgggaacgtccacattgccaacctgtgcaaagtggtcgccccggcacccagcaggtcgagacccgagcccgtggtcgtttgcctccgtggcaagtccggtcagggcaagagtttccttgcaaacgtgctcgcacaagcaatctctacccatttcactggcaggaccgattcagtttggtactgcccgcctgaccctgaccacttcgacggttacaaccaacagactgtcgttgtgatggacgatttgggccagaaccccgacggcaaagacttcaagtacttcgcccaaatggtttcaacaacggggttcatcccgcccatggcatcgcttgaggataaaggcaaacccttcaacagtaaggtcatcatagcaaccaccaacctgtactcgggcttcaccccgaggactatggtgtgccctgatgccctgaaccggaggtttcactttgacatcgacgtgagcgccaaggacgggtacaaaattaacaacaaattggacatcatcaaagcacttgaagatactcacaccaacccagtggcaatgtttcagtacgactgtgcccttctcaacggcatggctgttgaaatgaagagaatgcaacaagatatgttcaagcctcaaccaccccttcagaacgtgtaccaactggttcaagaggtgattgagcgggtggagctccacgagaaggtgtcgagccacccgattttcaaacagatctcaattccttcccaaaaatccgtgttgtacttcctcattgagaaaggacagcacgaggcagcaattgaattctttgagggcatggtgcacgactccatcaaggaggagctccggccgctcatccaacaaacctcatttgtgaaacgcgcttttaagcgcctgaaggaaaactttgagattgttgccctatgtctgaccctcctggccaacatagtgatcatgatccgcgaaactcgcaagagacagaagatggtggacgatgcagtgagtgagtacattgagagagcaaacatcaccaccgacgacaagactcttgatgaggcggaaaagaaccctctggaaaccagcggtgccagcaccgtcggcttcagagagagacctctcccaggccaaaaggcgcgtaatgacgagaactccgagcccgcccagcctgctgaagagcaaccacaagctgaaggaccctacgctggcccgatggagagaccagttaaagttaaagtgaaagcaaaagccccggtcgttaaggaaggaccttacgagggaccggtgaagaagcctgttgctttgaaagtgaaagctaagaacttgatcgtcactgagagtggtgccccaccgaccgacttgcaaaagttggtcatgggcaacaccaagcccgttgagctcatccttgacgggaagacggtagccatttgctgtgctactggagttttcggcactgcttacctcgtgcctcgtcatcttttcgcagaaaagtacgacaagatcatgttggacggcagagccatgacagatagtgactacagagtgtttgagtttgagattaaagtaaaaggacaggacatgctctcagacgctgcgctcatggtgctccaccgtgggaatcgcgtgagagacatcacgaaacactttcgtgacacagcaagaatgaagaaaggcacccccgtcgttggtgtgatcaacaacgccgatgtcgggagactgattttctctggtgaagcccttacctacaaggacattgtagtgtgcatggatggagacaccatgcctgggctctttgcctacaaagccgcaaccaaggctggttattgcggaggagccgtcctcgctaaggacggggctgacacgttcatcgttggcacccactccgctggaggcaatggcgttggatactgctcttgcgtttccaggtccatgcttctcaagatgaaggcacacgttgaccccgaaccacaccacgaggggttgattgttgacaccagagatgtggaagagcgcgttcacgtgatgcgcaaaaccaagcttgcacccaccgttgcgtacggtgtgttccgtcctgagttcgggcctgccgccttgtccaacaaggacccgcgcctgaacgacggtgttgtcctcgacgaagtcatcttctccaaacacaagggagacacaaagatgtctgaggaagacaaagcgctgttccgccgctgtgctgctgactacgcgtcacgcctgcacagcgtgttgggtacggcaaatgccccactgagcatctacgaggcaattaaaggcgttgatggactcgacgcaatggaaccagacaccgcacccggcctcccctgggcactccaggggaagcgccgtggcgcgctcatcgacttcgagaacggcactgttggacccgaagttgaggctgccttgaagctcatggagaaaagagaatacaagtttgcttgccaaaccttcctgaaggacgagattcgcccgatggagaaagtacgtgccggtaagactcgcattgtcgacgtcctacctgttgaacacatcctctacaccaggatgatgattggcagattttgtgcacaaatgcactcaaacaacggaccccaaattggctcggcggtcggttgtaaccctgatgttgattggcaaagatttggcacacacttcgcccaatacagaaacgtgtgggatgtggactattcggccttcgatgctaaccactgcagtgacgccatgaacatcatgtttgaggaagtgtttcgcacagaattcgggttccacccaaacgctgagtggatcctgaagactctcgtgaacacggaacacgcctatgagaacaaacgcatcactgttgaaggcgggatgccatctggttgttccgcaacaagcatcatcaacacaattttgaacaacatctacgtgctctacgctttgcgtagacactatgagggagttgagctggacacttacaccatgatctcttacggagacgatatcgtggtggcaagtgattacgatttggactttgaggctctcaagccccacttcaaatcccttggtcaaaccatcactccagctgacaaaagcgacaaaggttttgttcttggtcactccattactgatgtcactttcctcaaaagacacttccacatggattatggaactgggttttacaaacctgtgatggcctcaaagacccttgaggctatcctctcctttgcacgccgtgggaccatacaggagaagttgatctccgtggcaggactcgctgttcactctggaccagacgagtaccggcgtctcttcgagccctttcaaggcctcttcgagattccaagctacagatcactttacctgcgttgggtgaacgccgtgtgcggcgacgca

SEQ ID NO: 16 - protein, 2109 aa, Artificial Sequence
  Fusion protein:  Foot and Mouth Disease Virus (FMDV) and Bovine Rhinovirus Type 2 (BRV2)
GAGQSSPATGSQNQSGNTGSIINNYYMQQYQNSMDTQLGDNAISGGSNEGSTDTTSTHTTNTQNNDWFSKLASSAFTGLFGALLADKKTEETTLLEDRILTTRNGHTTSTTQSSVGVTHGYSTEEDHVAGPNTSGLETRVVQAERFYKKYLFDWTTDKAFGHLEKLELPSDHHGVFGHLVDSYAYMRNGWDVEVSAVGNQFNGGCLLVAMVPEWKEFDTREKYQLTLFPHQFISPRTNMTAHITVPYLGVNRYDQYKKHKPWTLVVMVVSPLTVNNTSAAQIKVYANIAPTYVHVAGELPSKEGIFPVACADGYGGLVTTDPKTADPAYGKVYNPPRTNYPGRFTNLLDVAEACPTFLCFDDGKPYVTTRTDDTRLLAKFDLSLAAKHMSNTYLSGIAQYYTQYSGTINLHFMFTGSTDSKARYMVAYIPPGVETPPDTPERAAHCIHAEWDTGLNSKFTFSIPYVSAADYAYTASDTAETINVQGWVCIYQITHGKAENDTLVVSVSAGKDFELRLPIDPRQQTTATGESADPVTTTVENYGGETQIQRRHHTDIGFIMDRFVKIQSLSPTHVIDLMQTHQHGLVGALLRAATYYFSDLEIVVRHEGNLTWVPNGAPESALLNTSNPTAYNKAPFTRLALPYTAPHRVLATVYNGTSKYAVGGSGRRGDMGSLAARVVKQLPASFNYGAIKADAIHELLVRMKRAELYCPRPLLAIEVSSQDRHKQKIIAPAKQLLNFDLLKLAGDVESNPGPFFFSDVRSNFSKLVDTINQMQEDMSTKHGPDFNRLVSAFEELATGVKAIRTGLDEAKPWYKLIKLLSRLSCMAAVAARSKDPVLVAIMLADTGLEILDSTFVVKKISDSLSSLFHVPAPVFSFGAPILLAGLVKVASSFFRSTPEDLERAEKQLKARDINDIFAILKNGEWLVKLILAIRDWIKAWIASEEKFVTTTDLVPSILEKQQDLNDPSKYKEAKEWLDNARQACLKSGNVHIANLCKVVAPAPSRSRPEPVVVCLRGKSGQGKSFLANVLAQAISTHFTGRTDSVWYCPPDPDHFDGYNQQTVVVMDDLGQNPDGKDFKYFAQMVSTTGFIPPMASLEDKGKPFNSKVIIATTNLYSGFTPRTMVCPDALNRRFHFDIDVSAKDGYKINNKLDIIKALEDTHTNPVAMFQYDCALLNGMAVEMKRMQQDMFKPQPPLQNVYQLVQEVIERVELHEKVSSHPIFKQISIPSQKSVLYFLIEKGQHEAAIEFFEGMVHDSIKEELRPLIQQTSFVKRAFKRLKENFEIVALCLTLLANIVIMIRETRKRQKMVDDAVSEYIERANITTDDKTLDEAEKNPLETSGASTVGFRERPLPGQKARNDENSEPAQPAEEQPQAEGPYAGPMERPVKVKVKAKAPVVKEGPYEGPVKKPVALKVKAKNLIVTESGAPPTDLQKLVMGNTKPVELILDGKTVAICCATGVFGTAYLVPRHLFAEKYDKIMLDGRAMTDSDYRVFEFEIKVKGQDMLSDAALMVLHRGNRVRDITKHFRDTARMKKGTPVVGVINNADVGRLIFSGEALTYKDIVVCMDGDTMPGLFAYKAATKAGYCGGAVLAKDGADTFIVGTHSAGGNGVGYCSCVSRSMLLKMKAHVDPEPHHEGLIVDTRDVEERVHVMRKTKLAPTVAYGVFRPEFGPAALSNKDPRLNDGVVLDEVIFSKHKGDTKMSEEDKALFRRCAADYASRLHSVLGTANAPLSIYEAIKGVDGLDAMEPDTAPGLPWALQGKRRGALIDFENGTVGPEVEAALKLMEKREYKFACQTFLKDEIRPMEKVRAGKTRIVDVLPVEHILYTRMMIGRFCAQMHSNNGPQIGSAVGCNPDVDWQRFGTHFAQYRNVWDVDYSAFDANHCSDAMNIMFEEVFRTEFGFHPNAEWILKTLVNTEHAYENKRITVEGGMPSGCSATSIINTILNNIYVLYALRRHYEGVELDTYTMISYGDDIVVASDYDLDFEALKPHFKSLGQTITPADKSDKGFVLGHSITDVTFLKRHFHMDYGTGFYKPVMASKTLEAILSFARRGTIQEKLISVAGLAVHSGPDEYRRLFEPFQGLFEIPSYRSLYLRWVNAVCGDA

SEQ ID NO: 17 - DNA, 6327 bp, Artificial Sequence
  Fusion nucleotide:  Foot and Mouth Disease Virus (FMDV) and Bovine Rhinovirus Type 2 (BRV2)
ggggccggccaatccagtccggcgaccggctcgcagaaccaatctggcaacactggcagcataattaacaactactacatgcagcaataccagaactccatggacacacagttgggagacaatgccatcagtggaggctccaacgagggctccacggacacaacttcaacacacacaaccaacactcaaaacaatgactggttctcgaagctcgccagttcagcttttaccggtctgttcggtgcactgctcgccgacaagaagacagaggaaacgacacttcttgaggaccgcatcctcaccacccgcaacgggcacaccacctcgacgacccaatcgagtgtgggtgtcacacacgggtactccacagaggaggaccacgttgctgggcccaacacatcgggcctggagacgcgagtggtgcaggcagagagattctacaaaaagtacttgtttgactggacaacggacaaggcatttggacacctggaaaagctggagctcccgtccgaccaccacggtgtctttggacacttggtggactcgtacgcctatatgagaaatggctgggatgttgaggtgtccgctgttggcaaccagttcaacggcgggtgcctcctggtggccatggtacctgaatggaaggaatttgacacacgggagaaataccaactcacccttttcccgcaccagtttattagccccagaactaacatgactgcccacatcacggtcccctaccttggtgtgaacaggtatgatcagtacaagaagcataagccctggacattggttgtcatggtcgtgtcgccacttacggtcaacaacactagtgcggcacaaatcaaggtctacgccaacatagctccgacctatgttcacgtggccggtgaactcccctcgaaagaggggattttcccggttgcatgtgcggacggttacggaggattggtgacgacagacccgaagacagctgaccctgcttatggcaaggtgtacaacccgcctaggactaactaccctgggcgcttcaccaacctgttggacgtggccgaagcgtgtcccactttcctctgctttgacgacgggaaaccgtacgtcaccacgcggacggatgacacccgacttttggccaagtttgacctttcccttgccgcaaaacatatgtccaacacatacctgtcagggattgctcagtactacacacagtactctggcaccatcaatttgcatttcatgttcacaggttccactgattcaaaggcccgatacatggtggcctacatcccacctggggtggagacaccaccggacacacctgaaagggctgcccactgcattcacgctgaatgggacactggactaaactccaaattcactttctcaatcccgtacgtatccgccgcggattacgcgtacacagcgtctgacacggcagaaacaatcaacgtacagggatgggtctgcatctaccaaattacacacgggaaggctgaaaatgacaccttggtcgtgtcggttagcgccggcaaagactttgagttgcgcctcccgattgacccccgccagcagaccaccgctaccggggaatcagcagacccggtcaccaccaccgtggagaactacggcggtgagacacaaatccagagacgtcaccacacggacattggtttcatcatggacagatttgtgaagatccaaagcttgagcccaacacatgtcattgacctcatgcagactcaccaacacggtctggtgggtgccttgctgcgtgcagccacgtactacttttctgacctggaaattgttgtacggcacgaaggcaatctgacctgggtgcccaacggcgcccctgaatcagccctgttgaacaccagcaaccccactgcctacaacaaggcaccattcacgagactcgctctcccctacactgcgccgcaccgtgtgctggcaacagtgtacaacgggacgagtaagtatgctgtgggtggttcaggcagaagaggcgacatggggtctctcgcggcgcgagtcgtgaaacagcttcctgcttcatttaactacggtgcaatcaaggccgacgccatccacgaacttctcgtgcgcatgaaacgggccgagctctactgccccagaccgctgttggcaatagaggtgtcttcgcaagacaggcacaagcaaaagatcattgcaccagcaaagcagcttctgaattttgacctgcttaagctagccggagacgttgagtccaaccctgggcccttcttcttctccgacgttaggtcaaacttttccaagctggtagacacaatcaaccagatgcaggaagacatgtccacaaagcacggacctgactttaaccggttggtgtccgcttttgaggagttggccactggagtgaaagccatcaggaccggtcttgacgaggccaagccctggtacaagcttatcaagctcctgagccgcctgtcgtgcatggccgctgtggcagcacggtcaaaggacccagtccttgtggccatcatgctggctgacaccggtctcgagattctggacagcaccttcgtcgtgaagaagatctccgactcgctctccagtctcttccacgtgccggcccccgtcttcagtttcggagccccgattctgttagccgggttggtcaaggtcgcctcgagtttcttccggtccacgcccgaagaccttgagagagcagagaaacagctcaaagcacgtgacatcaacgacattttcgccattctcaagaacggcgagtggctggtcaaattgatccttgccatccgcgactggatcaaggcatggatagcctcagaagaaaagtttgtcaccacgacagacttggtacctagcatccttgaaaaacagcaggacctcaacgacccaagcaagtacaaggaagccaaggagtggctcgacaacgcgcgccaagcgtgtttgaagagcgggaacgtccacattgccaacctgtgcaaagtggtcgccccggcacccagcaggtcgagacccgagcccgtggtcgtttgcctccgtggcaagtccggtcagggcaagagtttccttgcaaacgtgctcgcacaagcaatctctacccatttcactggcaggaccgattcagtttggtactgcccgcctgaccctgaccacttcgacggttacaaccaacagactgtcgttgtgatggacgatttgggccagaaccccgacggcaaagacttcaagtacttcgcccaaatggtttcaacaacggggttcatcccgcccatggcatcgcttgaggataaaggcaaacccttcaacagtaaggtcatcatagcaaccaccaacctgtactcgggcttcaccccgaggactatggtgtgccctgatgccctgaaccggaggtttcactttgacatcgacgtgagcgccaaggacgggtacaaaattaacaacaaattggacatcatcaaagcacttgaagatactcacaccaacccagtggcaatgtttcagtacgactgtgcccttctcaacggcatggctgttgaaatgaagagaatgcaacaagatatgttcaagcctcaaccaccccttcagaacgtgtaccaactggttcaagaggtgattgagcgggtggagctccacgagaaggtgtcgagccacccgattttcaaacagatctcaattccttcccaaaaatccgtgttgtacttcctcattgagaaaggacagcacgaggcagcaattgaattctttgagggcatggtgcacgactccatcaaggaggagctccggccgctcatccaacaaacctcatttgtgaaacgcgcttttaagcgcctgaaggaaaactttgagattgttgccctatgtctgaccctcctggccaacatagtgatcatgatccgcgaaactcgcaagagacagaagatggtggacgatgcagtgagtgagtacattgagagagcaaacatcaccaccgacgacaagactcttgatgaggcggaaaagaaccctctggaaaccagcggtgccagcaccgtcggcttcagagagagacctctcccaggccaaaaggcgcgtaatgacgagaactccgagcccgcccagcctgctgaagagcaaccacaagctgaaggaccctacgctggcccgatggagagacagaaaccactgaaagtgaaagcaaaagccccggtcgttaaggaaggaccttacgagggaccggtgaagaagcctgttgctttgaaagtgaaagctaagaacttgatcgtcactgagagtggtgccccaccgaccgacttgcaaaagttggtcatgggcaacaccaagcccgttgagctcatccttgacgggaagacggtagccatttgctgtgctactggagttttcggcactgcttacctcgtgcctcgtcatcttttcgcagaaaagtacgacaagatcatgttggacggcagagccatgacagatagtgactacagagtgtttgagtttgagattaaagtaaaaggacaggacatgctctcagacgctgcgctcatggtgctccaccgtgggaatcgcgtgagagacatcacgaaacactttcgtgacacagcaagaatgaagaaaggcacccccgtcgttggtgtgatcaacaacgccgatgtcgggagactgattttctctggtgaagcccttacctacaaggacattgtagtgtgcatggatggagacaccatgcctgggctctttgcctacaaagccgcaaccaaggctggttattgcggaggagccgtcctcgctaaggacggggctgacacgttcatcgttggcacccactccgctggaggcaatggcgttggatactgctcttgcgtttccaggtccatgcttctcaagatgaaggcacacgttgaccccgaaccacaccacgaggggttgattgttgacaccagagatgtggaagagcgcgttcacgtgatgcgcaaaaccaagcttgcacccaccgttgcgtacggtgtgttccgtcctgagttcgggcctgccgccttgtccaacaaggacccgcgcctgaacgacggtgttgtcctcgacgaagtcatcttctccaaacacaagggagacacaaagatgtctgaggaagacaaagcgctgttccgccgctgtgctgctgactacgcgtcacgcctgcacagcgtgttgggtacggcaaatgccccactgagcatctacgaggcaattaaaggcgttgatggactcgacgcaatggaaccagacaccgcacccggcctcccctgggcactccaggggaagcgccgtggcgcgctcatcgacttcgagaacggcactgttggacccgaagttgaggctgccttgaagctcatggagaaaagagaatacaagtttgcttgccaaaccttcctgaaggacgagattcgcccgatggagaaagtacgtgccggtaagactcgcattgtcgacgtcctacctgttgaacacatcctctacaccaggatgatgattggcagattttgtgcacaaatgcactcaaacaacggaccccaaattggctcggcggtcggttgtaaccctgatgttgattggcaaagatttggcacacacttcgcccaatacagaaacgtgtgggatgtggactattcggccttcgatgctaaccactgcagtgacgccatgaacatcatgtttgaggaagtgtttcgcacagaattcgggttccacccaaacgctgagtggatcctgaagactctcgtgaacacggaacacgcctatgagaacaaacgcatcactgttgaaggcgggatgccatctggttgttccgcaacaagcatcatcaacacaattttgaacaacatctacgtgctctacgctttgcgtagacactatgagggagttgagctggacacttacaccatgatctcttacggagacgatatcgtggtggcaagtgattacgatttggactttgaggctctcaagccccacttcaaatcccttggtcaaaccatcactccagctgacaaaagcgacaaaggttttgttcttggtcactccattactgatgtcactttcctcaaaagacacttccacatggattatggaactgggttttacaaacctgtgatggcctcaaagacccttgaggctatcctctcctttgcacgccgtgggaccatacaggagaagttgatctccgtggcaggactcgctgttcactctggaccagacgagtaccggcgtctcttcgagccctttcaaggcctcttcgagattccaagctacagatcactttacctgcgttgggtgaacgccgtgtgcggcgacgca

SEQ ID NO: 18 - protein, 2109 aa, Artificial Sequence
  Fusion protein:  Foot and Mouth Disease Virus (FMDV) and Bovine Rhinovirus Type 2 (BRV2)
GAGQSSPATGSQNQSGNTGSIINNYYMQQYQNSMDTQLGDNAISGGSNEGSTDTTSTHTTNTQNNDWFSKLASSAFTGLFGALLADKKTEETTLLEDRILTTRNGHTTSTTQSSVGVTHGYSTEEDHVAGPNTSGLETRVVQAERFYKKYLFDWTTDKAFGHLEKLELPSDHHGVFGHLVDSYAYMRNGWDVEVSAVGNQFNGGCLLVAMVPEWKEFDTREKYQLTLFPHQFISPRTNMTAHITVPYLGVNRYDQYKKHKPWTLVVMVVSPLTVNNTSAAQIKVYANIAPTYVHVAGELPSKEGIFPVACADGYGGLVTTDPKTADPAYGKVYNPPRTNYPGRFTNLLDVAEACPTFLCFDDGKPYVTTRTDDTRLLAKFDLSLAAKHMSNTYLSGIAQYYTQYSGTINLHFMFTGSTDSKARYMVAYIPPGVETPPDTPERAAHCIHAEWDTGLNSKFTFSIPYVSAADYAYTASDTAETINVQGWVCIYQITHGKAENDTLVVSVSAGKDFELRLPIDPRQQTTATGESADPVTTTVENYGGETQIQRRHHTDIGFIMDRFVKIQSLSPTHVIDLMQTHQHGLVGALLRAATYYFSDLEIVVRHEGNLTWVPNGAPESALLNTSNPTAYNKAPFTRLALPYTAPHRVLATVYNGTSKYAVGGSGRRGDMGSLAARVVKQLPASFNYGAIKADAIHELLVRMKRAELYCPRPLLAIEVSSQDRHKQKIIAPAKQLLNFDLLKLAGDVESNPGPFFFSDVRSNFSKLVDTINQMQEDMSTKHGPDFNRLVSAFEELATGVKAIRTGLDEAKPWYKLIKLLSRLSCMAAVAARSKDPVLVAIMLADTGLEILDSTFVVKKISDSLSSLFHVPAPVFSFGAPILLAGLVKVASSFFRSTPEDLERAEKQLKARDINDIFAILKNGEWLVKLILAIRDWIKAWIASEEKFVTTTDLVPSILEKQQDLNDPSKYKEAKEWLDNARQACLKSGNVHIANLCKVVAPAPSRSRPEPVVVCLRGKSGQGKSFLANVLAQAISTHFTGRTDSVWYCPPDPDHFDGYNQQTVVVMDDLGQNPDGKDFKYFAQMVSTTGFIPPMASLEDKGKPFNSKVIIATTNLYSGFTPRTMVCPDALNRRFHFDIDVSAKDGYKINNKLDIIKALEDTHTNPVAMFQYDCALLNGMAVEMKRMQQDMFKPQPPLQNVYQLVQEVIERVELHEKVSSHPIFKQISIPSQKSVLYFLIEKGQHEAAIEFFEGMVHDSIKEELRPLIQQTSFVKRAFKRLKENFEIVALCLTLLANIVIMIRETRKRQKMVDDAVSEYIERANITTDDKTLDEAEKNPLETSGASTVGFRERPLPGQKARNDENSEPAQPAEEQPQAEGPYAGPMERQKPLKVKAKAPVVKEGPYEGPVKKPVALKVKAKNLIVTESGAPPTDLQKLVMGNTKPVELILDGKTVAICCATGVFGTAYLVPRHLFAEKYDKIMLDGRAMTDSDYRVFEFEIKVKGQDMLSDAALMVLHRGNRVRDITKHFRDTARMKKGTPVVGVINNADVGRLIFSGEALTYKDIVVCMDGDTMPGLFAYKAATKAGYCGGAVLAKDGADTFIVGTHSAGGNGVGYCSCVSRSMLLKMKAHVDPEPHHEGLIVDTRDVEERVHVMRKTKLAPTVAYGVFRPEFGPAALSNKDPRLNDGVVLDEVIFSKHKGDTKMSEEDKALFRRCAADYASRLHSVLGTANAPLSIYEAIKGVDGLDAMEPDTAPGLPWALQGKRRGALIDFENGTVGPEVEAALKLMEKREYKFACQTFLKDEIRPMEKVRAGKTRIVDVLPVEHILYTRMMIGRFCAQMHSNNGPQIGSAVGCNPDVDWQRFGTHFAQYRNVWDVDYSAFDANHCSDAMNIMFEEVFRTEFGFHPNAEWILKTLVNTEHAYENKRITVEGGMPSGCSATSIINTILNNIYVLYALRRHYEGVELDTYTMISYGDDIVVASDYDLDFEALKPHFKSLGQTITPADKSDKGFVLGHSITDVTFLKRHFHMDYGTGFYKPVMASKTLEAILSFARRGTIQEKLISVAGLAVHSGPDEYRRLFEPFQGLFEIPSYRSLYLRWVNAVCGDA

SEQ ID NO: 19 - protein, 40 aa, Artificial Sequence
  Foot-and-mouth disease virus
GLIVDTRDVEERVHVMRKTKLAPTVAHGVFNPEFGPAALS

SEQ ID NO: 20 - protein, 40 aa, Artificial Sequence
  Foot-and-mouth disease virus
GLIVDTRDVEERVHVMRKTKLAPTVAYGVFRPEFGPAALS

SEQ ID NO: 21 - protein, 24 aa, Artificial Sequence
  Foot-and-mouth disease virus
GPYAGPMERQKPLKVRAKAPVVKE

SEQ ID NO: 22 - protein, 24 aa, Artificial Sequence
  Foot-and-mouth disease virus
GPYAGPMEPVKVLKVRAKAPVVKE

SEQ ID NO: 23 - DNA, 7589 bp, Artificial Sequence
  Fusion nucleotide:  Foot and Mouth Disease Virus (FMDV) and Bovine Rhinovirus Type 2 (BRV2)
ttgaaagggggcgctagggtctcacccctagcatgccaacgacagtccccgcgttgcactccacactcacgttgtgcgtgcgcggagctcgatggactatcgttcacccacctacagctggactcacggcaccgtgtggccacttggctggattgtgcggacgaacaccgcttgcgcttctcgcgtgaccggttagtactctcaccaccttccgcccacttggttgttagcgctgtcttgggcactcctgttgggggccgttcgacgctccgcgagtttccccgcacggcaactacggtgatggggccgtaccgcgcgggctgatcgcctggtgtgcttcggctgtcacccgaagcctacctttcaccccccccccccccccccccccccccccccccccccccccctaagttctaccgtcgttcccgacgtaaagggatgtaaccacaagcttactaccgcctttcccggcgttaaagggatgtaaccacaagacttaccttcacccggaagtaaaacggcaacttcacacagttttgcccgttttcatgagaaatgggacgtctgcgcacgaaacgcgccgtcgcttgaggaggacttgtacaaacacgatctaagcaggtttccccaactgacacaaaccgtgcaatttgaaactccgcctgggctttccaggtctagaggggtgacgctttgtactgtgtttgactccacgttcgatccactggcgagtgttagtaacaacactgctgcttcgtagcggagcatgacggccgtgggacccccccccttggtaacaaggacccacggggccaaaagccacgtccgaatggacccgtcatgtgtgcaaacccagcacagtagctttgttgtgaaactcactttaaagtgacattgatactggtactcaagcactggtgacaggctaaggatgcccttcaggtaccccgaggtaacacgtgacactcgggatctgagaaggggaccggggcttctataaaagcgcccggtttaaaaagcttctatgtctgaataggtgaccggaggccggcacctttcttttaattacactggacttatgaacacaactgattgttttatcgctttggtacacgctatcagagagatcagagcatttttcctaccacgagccacaggaatgggggccggccaatccagtccggcaaccgggtcacagaaccaatctggcaacactggaagcatcattaacaactactacatgcaacagtaccagaattccatggacacacagcttggtgacaacgctattagcggaggttccaacgaaggttccacggataccacttccacacacacaaacaacacccaaaacaacgactggttctcgcgcctggcaagttctgcattcagtggtctctttggtgcacttttggctgacaagaagacagaagagacaactctgcttgaagaccgcattctcaccaccaggaacggccacacaacatcgacgacacagtcgagcgttggcgtaacatacggttacgctgtggccgaggacgcggtgtctggacccaatacctcgggtctagagactcgtgttcaacaggcagaacggtttttcaagaaacacctgtttgactggacaccgaacttggcatttggacactgttactacctggaacttcccactgaacacaaaggcgtgtacggcagtctcatgggctcgtacgcctacatgagaaatggatgggacatagaggtgactgctgttggaaaccaattcaacggtggttgtctccttgtcgcgctcgtgccagagctgaaggaactcgacacgcgacagaagtaccagctgaccctctttccccaccagttcatcaacccacgcaccaacatgacggcccacatcaacgtgccgtacgtgggtatcaacaggtacgaccagtacgccctccacaagccgtggacgcttgttgtgatggtggtagccccactcaccgtcaaaactggtggttctgaacagatcaaggtttacatgaatgcagcgccaacctacgtgcatgtggcgggagagctgccctcgaaagagggaatagttcccgtcgcgtgtgcggacggttacggcaacatggtgaccacggacccgaagacggccgatccagtttacgggaaagtgttcaacccccccaggacaaacctccctgggcgcttcacgaacttccttgatgttgcggaggcatgtccaactttcctccgctttggagaagtaccatttgtgaagacggtgaactctggtgaccgcttgctggccaagttcgacgtgtccctcgctgcagggcacatgtccaacacctacttggctggcctggcgcagtactacacacagtacagcggcaccatgaacgtccacttcatgttcaccgggcccacggatgctaaagcccgatacatggtggcttatgtcccccctggcatgacaccgcccacggaccctgagcacgccgcacactgcattcactctgagtgggatactggtcttaactctaagtttaccttttccataccttacctctctgctgctgactatgcctacactgcttctgacgtggcggagaccacgagtgtgcagggatgggtgtgtatctatcagatcacccacggcaaggctgagggagacgcactggtcgtttctgtcagcgccggcaaagactttgagtttcgcttgcctgttgacgcacgccagcaaaccaccaccactggcgaatcagcagatccagtcacaaccacggttgagaactatggaggagagactcagacagccagacggcttcacactgacgtcgccttcattcttgacaggtttgtgaaactcactgctcccaagaacatccaaaccctcgatctcatgcagatcccctcacacacgctggttggagcactacttcgttctgcgacgtactacttctcagacctggaggtcgcgcttgtccacacaggcccggtcacctgggtgcccaacggcgcgcccaaggatgctctaaacaaccagaccaacccaactgcctatcagaagcaacccatcacccgcctggcactcccctacaccgccccccatcgtgtgctggcaacagtgtacaacgggaagacggcgtacggggaaacgacctcaaggcgcggcgacatggcggccctcgcacaaaggttgagcgctcggctgcccacctccttcaactacggcgccgtgaaggccgacaccatcactgagcttttgatccgcatgaagcgcgcggagacatattgccctaggcctttactagcccttgacaccactcaggaccgccgcaaacaggagatcattgcacctgagaagcagcttctgaattttgacctgcttaagctagccggagacgttgagtccaaccctgggcccttcttcttctccgacgttaggtcaaacttttccaagctggtagacacaatcaaccagatgcaggaagacatgtccacaaagcacggacctgactttaaccggttggtgtccgcttttgaggagttggccactggagtgaaagccatcaggaccggtcttgacgaggccaagccctggtacaagcttatcaagctcctgagccgcctgtcgtgcatggccgctgtggcagcacggtcaaaggacccagtccttgtggccatcatgctggctgacaccggtctcgagattctggacagcaccttcgtcgtgaagaagatctccgactcgctctccagtctcttccacgtgccggcccccgtcttcagtttcggagccccgattctgttagccgggttggtcaaggtcgcctcgagtttcttccggtccacgcccgaagaccttgagagagcagagaaacagctcaaagcacgtgacatcaacgacattttcgccattctcaagaacggcgagtggctggtcaaattgatccttgccatccgcgactggatcaaggcatggatagcctcagaagaaaagtttgtcaccacgacagacttggtacctagcatccttgaaaaacagcaggacctcaacgacccaagcaagtacaaggaagccaaggagtggctcgacaacgcgcgccaagcgtgtttgaagagcgggaacgtccacattgccaacctgtgcaaagtggtcgccccggcacccagcaggtcgagacccgagcccgtggtcgtttgcctccgtggcaagtccggtcagggcaagagtttccttgcaaacgtgctcgcacaagcaatctctacccatttcactggcaggaccgattcagtttggtactgcccgcctgaccctgaccacttcgacggttacaaccaacagactgtcgttgtgatggacgatttgggccagaaccccgacggcaaagacttcaagtacttcgcccaaatggtttcaacaacggggttcatcccgcccatggcatcgcttgaggataaaggcaaacccttcaacagtaaggtcatcatagcaaccaccaacctgtactcgggcttcaccccgaggactatggtgtgccctgatgccctgaaccggaggtttcactttgacatcgacgtgagcgccaaggacgggtacaaaattaacaacaaattggacatcatcaaagcacttgaagatactcacaccaacccagtggcaatgtttcagtacgactgtgcccttctcaacggcatggctgttgaaatgaagagaatgcaacaagatatgttcaagcctcaaccaccccttcagaacgtgtaccaactggttcaagaggtgattgagcgggtggagctccacgagaaggtgtcgagccacccgattttcaaacagatctcaattccttcccaaaaatccgtgttgtacttcctcattgagaaaggacagcacgaggcagcaattgaattctttgagggcatggtgcacgactccatcaaggaggagctccggccgctcatccaacaaacctcatttgtgaaacgcgcttttaagcgcctgaaggaaaactttgagattgttgccctatgtctgaccctcctggccaacatagtgatcatgatccgcgaaactcgcaagagacagaagatggtggacgatgcagtgagtgagtacattgagagagcaaacatcaccaccgacgacaagactcttgatgaggcggaaaagaaccctctggaaaccagcggtgccagcaccgtcggcttcagagagagacctctcccaggccaaaaggcgcgtaatgacgagaactccgagcccgcccagcctgctgaagagcaaccacaagctgaaggaccctacgctggcccgatggagagaccagttaaagttaaagtgaaagcaaaagccccggtcgttaaggaaggaccttacgagggaccggtgaagaagcctgttgctttgaaagtgaaagctaagaacttgatcgtcactgagagtggtgccccaccgaccgacttgcaaaagttggtcatgggcaacaccaagcccgttgagctcatccttgacgggaagacggtagccatttgctgtgctactggagttttcggcactgcttacctcgtgcctcgtcatcttttcgcagaaaagtacgacaagatcatgttggacggcagagccatgacagatagtgactacagagtgtttgagtttgagattaaagtaaaaggacaggacatgctctcagacgctgcgctcatggtgctccaccgtgggaatcgcgtgagagacatcacgaaacactttcgtgacacagcaagaatgaagaaaggcacccccgtcgttggtgtgatcaacaacgccgatgtcgggagactgattttctctggtgaagcccttacctacaaggacattgtagtgtgcatggatggagacaccatgcctgggctctttgcctacaaagccgcaaccaaggctggttattgcggaggagccgtcctcgctaaggacggggctgacacgttcatcgttggcacccactccgctggaggcaatggcgttggatactgctcttgcgtttccaggtccatgcttctcaagatgaaggcacacgttgaccccgaaccacaccacgaggggttgattgttgacaccagagatgtggaagagcgcgttcacgtgatgcgcaaaaccaagcttgcacccaccgttgcgtacggtgtgttccgtcctgagttcgggcctgccgccttgtccaacaaggacccgcgcctgaacgacggtgttgtcctcgacgaagtcatcttctccaaacacaagggagacacaaagatgtctgaggaagacaaagcgctgttccgccgctgtgctgctgactacgcgtcacgcctgcacagcgtgttgggtacggcaaatgccccactgagcatctacgaggcaattaaaggcgttgatggactcgacgcaatggaaccagacaccgcacccggcctcccctgggcactccaggggaagcgccgtggcgcgctcatcgacttcgagaacggcactgttggacccgaagttgaggctgccttgaagctcatggagaaaagagaatacaagtttgcttgccaaaccttcctgaaggacgagattcgcccgatggagaaagtacgtgccggtaagactcgcattgtcgacgtcctacctgttgaacacatcctctacaccaggatgatgattggcagattttgtgcacaaatgcactcaaacaacggaccccaaattggctcggcggtcggttgtaaccctgatgttgattggcaaagatttggcacacacttcgcccaatacagaaacgtgtgggatgtggactattcggccttcgatgctaaccactgcagtgacgccatgaacatcatgtttgaggaagtgtttcgcacagaattcgggttccacccaaacgctgagtggatcctgaagactctcgtgaacacggaacacgcctatgagaacaaacgcatcactgttgaaggcgggatgccatctggttgttccgcaacaagcatcatcaacacaattttgaacaacatctacgtgctctacgctttgcgtagacactatgagggagttgagctggacacttacaccatgatctcttacggagacgatatcgtggtggcaagtgattacgatttggactttgaggctctcaagccccacttcaaatcccttggtcaaaccatcactccagctgacaaaagcgacaaaggttttgttcttggtcactccattactgatgtcactttcctcaaaagacacttccacatggattatggaactgggttttacaaacctgtgatggcctcaaagacccttgaggctatcctctcctttgcacgccgtgggaccatacaggagaagttgatctccgtggcaggactcgctgttcactctggaccagacgagtaccggcgtctcttcgagccctttcaaggcctcttcgagattccaagctacagatcactttacctgcgttgggtgaacgccgtgtgcggcgacgcataatccctcagagactacattggcatactgtttctgaggcgcgcgacgccgtaggagtgaaaagcctgaaagggcttttcccgcttcctattccaaaaaaaaaaaaaaaaaa

SEQ ID NO: 24 - DNA, 7600 bp, Artificial Sequence
  Fusion nucleotide:  Foot and Mouth Disease Virus (FMDV) and Bovine Rhinovirus Type 2 (BRV2)
ttgaaagggggcgctagggtctcacccctagcatgccaacgacagtccccgcgttgcactccacactcacgttgtgcgtgcgcggagctcgatggactatcgttcacccacctacagctggactcacggcaccgtgtggccacttggctggattgtgcggacgaacaccgcttgcgcttctcgcgtgaccggttagtactctcaccaccttccgcccacttggttgttagcgctgtcttgggcactcctgttgggggccgttcgacgctccgcgagtttccccgcacggcaactacggtgatggggccgtaccgcgcgggctgatcgcctggtgtgcttcggctgtcacccgaagcctacctttcaccccccccccccccccccccccccccccccccccccccccctaagttctaccgtcgttcccgacgtaaagggatgtaaccacaagcttactaccgcctttcccggcgttaaagggatgtaaccacaagacttaccttcacccggaagtaaaacggcaacttcacacagttttgcccgttttcatgagaaatgggacgtctgcgcacgaaacgcgccgtcgcttgaggaggacttgtacaaacacgatctaagcaggtttccccaactgacacaaaccgtgcaatttgaaactccgcctgggctttccaggtctagaggggtgacgctttgtactgtgtttgactccacgttcgatccactggcgagtgttagtaacaacactgctgcttcgtagcggagcatgacggccgtgggacccccccccttggtaacaaggacccacggggccaaaagccacgtccgaatggacccgtcatgtgtgcaaacccagcacagtagctttgttgtgaaactcactttaaagtgacattgatactggtactcaagcactggtgacaggctaaggatgcccttcaggtaccccgaggtaacacgtgacactcgggatctgagaaggggaccggggcttctataaaagcgcccggtttaaaaagcttctatgtctgaataggtgaccggaggccggcacctttcttttaattacactggacttatgaacacaactgattgttttatcgctttggtacacgctatcagagagatcagagcatttttcctaccacgagccacaggaatgggggccggccaatccagtccggcaaccgggtcacaaaaccaatcaggcaacactggtagtatcatcaacaactactacatgcagcagtaccagaactccatggatacacaacttggcgacaacgccattagcggtggttccaacgagggctccactgacactacctccacacacacaaccaacacacagaacaatgactggttttcaaagctggccagttctgccttcagcggtctcttcggcgctcttctcgctgacaaaaagacagaggagactaccctcctggaggaccgcatccttaccacccgcaacggacacaccacctcgacaacccagtcgagtgtgggtgtcacctacgggtactccactggtgaagaccacgtctctggacctaacacatctggcctggagacgcgagtggtacaggcagagagattcttcaagaaacacttgtttgattggacaactgataaagcttttggacacctggaaaaactggaactccccaccgaacacaagggtgtctacgggcacttggtggactctttcgcatacatgagaaatggctgggacgtggaggtgaccgccgttggcaaccagttcaacggtgggtgtctcctggtggccatggtacctgagtggaaagagtttacccctcgtgagaaataccagctcaccctgtttccacaccaatttatcaaccccagaaccaacatgacagcccacatcacggtcccgtaccttggtgtcaataggtatgaccagtacaaacagcacaaaccctggacactggtcgtgatggtggtttcgccactgaccaccagcagcattggggcctcacagattaaggtctacgccaacattgccccaaccttcgttcacgtggccggcgagctcccatcgaaagaagggatcgtgccggttgcttgtacagacgggtacggtggcctggtgacaacagacccgaaaacagctgaccctgtttatggtatggtgtacaacccgcccagaaccaactaccctgggcgctttacaaacttgttggacgtggccgaggcttgcccgaccttcctctgttttgacgacgggaaaccgtacgttgtgacaaggacggacgaccaacgcctcctggccaagtttgacgtttcccttgctgcaaagcacatgtcaaacacctacctctcagggatagcacagtactacacgcagtactctggcactatcaatctgcatttcatgttcactggctctactgaatcaaaggcccggtacatggtggcgtacattccacctggcatggacaacccaccggacacacctgagaaggctgcacattgcatccacgccgagtgggacaccgggctgaactccaaatttactttttctatcccgtacgtgtctgctgcagactacgcatacactgcgtctgacgtggcagaaacaacaaacgtacaggggtgggtctgcatataccaaatcactcacgggaaggctgaacaggacactctggtcgtgtcggtcagcgccggcaaggactttgaactgcgcctcccaattgacccccgcacgcaaaccaccactgccggggagtcagcagaccctgtcaccaccaccgttgagaactacggtggtgagacacaggctcagcgacgtcagcacactgacgtcggcttcatcatggacaggtttgcgaaaatcagccccgtgagccccacgcacgtcattgacctcatgcaaacacaccaacacgcgttggtgggtgcccttttgcgtgcagccacgtactacttctccgatctggagattgtggtgcgtcatgatggcaacttgacgtgggtgcccaatggagcacctgtagaagccttggccaacacaagcaaccccaccgcctaccacaagcagccatttacgagacttgcgctcccttacaccgcgccgcaccgagtgttggcaacagtgtataacggagtaagcaagtactctacaactggtaatggcagaaggggtgacctggggcctcttgcggcgcgggtcgccgcacagctccccagctctttcaattttggtgcaattcgggccacgaccgtccacgagcttctcgtgcgcatgaaacgtgccgagctctactgtcccaggcctctgctggcagtggaagtgttgtcgcaggacagacacaagcaaaagatcattgcacctgcaaagcaacttctgaattttgacctgcttaagctagccggagacgttgagtccaaccctgggcccttcttcttctccgacgttaggtcaaacttttccaagctggtagacacaatcaaccagatgcaggaagacatgtccacaaagcacggacctgactttaaccggttggtgtccgcttttgaggagttggccactggagtgaaagccatcaggaccggtcttgacgaggccaagccctggtacaagcttatcaagctcctgagccgcctgtcgtgcatggccgctgtggcagcacggtcaaaggacccagtccttgtggccatcatgctggctgacaccggtctcgagattctggacagcaccttcgtcgtgaagaagatctccgactcgctctccagtctcttccacgtgccggcccccgtcttcagtttcggagccccgattctgttagccgggttggtcaaggtcgcctcgagtttcttccggtccacgcccgaagaccttgagagagcagagaaacagctcaaagcacgtgacatcaacgacattttcgccattctcaagaacggcgagtggctggtcaaattgatccttgccatccgcgactggatcaaggcatggatagcctcagaagaaaagtttgtcaccacgacagacttggtacctagcatccttgaaaaacagcaggacctcaacgacccaagcaagtacaaggaagccaaggagtggctcgacaacgcgcgccaagcgtgtttgaagagcgggaacgtccacattgccaacctgtgcaaagtggtcgccccggcacccagcaggtcgagacccgagcccgtggtcgtttgcctccgtggcaagtccggtcagggcaagagtttccttgcaaacgtgctcgcacaagcaatctctacccatttcactggcaggaccgattcagtttggtactgcccgcctgaccctgaccacttcgacggttacaaccaacagactgtcgttgtgatggacgatttgggccagaaccccgacggcaaagacttcaagtacttcgcccaaatggtttcaacaacggggttcatcccgcccatggcatcgcttgaggataaaggcaaacccttcaacagtaaggtcatcatagcaaccaccaacctgtactcgggcttcaccccgaggactatggtgtgccctgatgccctgaaccggaggtttcactttgacatcgacgtgagcgccaaggacgggtacaaaattaacaacaaattggacatcatcaaagcacttgaagatactcacaccaacccagtggcaatgtttcagtacgactgtgcccttctcaacggcatggctgttgaaatgaagagaatgcaacaagatatgttcaagcctcaaccaccccttcagaacgtgtaccaactggttcaagaggtgattgagcgggtggagctccacgagaaggtgtcgagccacccgattttcaaacagatctcaattccttcccaaaaatccgtgttgtacttcctcattgagaaaggacagcacgaggcagcaattgaattctttgagggcatggtgcacgactccatcaaggaggagctccggccgctcatccaacaaacctcatttgtgaaacgcgcttttaagcgcctgaaggaaaactttgagattgttgccctatgtctgaccctcctggccaacatagtgatcatgatccgcgaaactcgcaagagacagcagatggtggacgatgcagtgagtgagtacattgagagagcaaacatcaccaccgacgacaagactcttgatgaggcggaaaagaaccctctggaaaccagcggtgccagcaccgtcggcttcagagagagacctctcccaggccaaaaggcgcgtaatgacgagaactccgagcccgcccagcctgctgaagagcaaccacaagctgaaggaccctacgctggcccgatggagagaccagttaaagttaaagtgaaagcaaaagccccggtcgttaaggaaggaccttacgagggaccggtgaagaagcctgttgctttgaaagtgaaagctaagaacttgatcgtcactgagagtggtgccccaccgaccgacttgcaaaagttggtcatgggcaacaccaagcccgttgagctcatccttgacgggaagacggtagccatttgctgtgctactggagttttcggcactgcttacctcgtgcctcgtcatcttttcgcagaaaagtacgacaagatcatgttggacggcagagccatgacagatagtgactacagagtgtttgagtttgagattaaagtaaaaggacaggacatgctctcagacgctgcgctcatggtgctccaccgtgggaatcgcgtgagagacatcacgaaacactttcgtgacacagcaagaatgaagaaaggcacccccgtcgttggtgtgatcaacaacgccgatgtcgggagactgattttctctggtgaagcccttacctacaaggacattgtagtgtgcatggatggagacaccatgcctgggctctttgcctacaaagccgcaaccaaggctggttattgcggaggagccgtcctcgctaaggacggggctgacacgttcatcgttggcacccactccgctggaggcaatggcgttggatactgctcttgcgtttccaggtccatgcttctcaagatgaaggcacacgttgaccccgaaccacaccacgaggggttgattgttgacaccagagatgtggaagagcgcgttcacgtgatgcgcaaaaccaagcttgcacccaccgttgcgtacggtgtgttccgtcctgagttcgggcctgccgccttgtccaacaaggacccgcgcctgaacgacggtgttgtcctcgacgaagtcatcttctccaaacacaagggagacacaaagatgtctgaggaagacaaagcgctgttccgccgctgtgctgctgactacgcgtcacgcctgcacagcgtgttgggtacggcaaatgccccactgagcatctacgaggcaattaaaggcgttgatggactcgacgcaatggaaccagacaccgcacccggcctcccctgggcactccaggggaagcgccgtggcgcgctcatcgacttcgagaacggcactgttggacccgaagttgaggctgccttgaagctcatggagaaaagagaatacaagtttgcttgccaaaccttcctgaaggacgagattcgcccgatggagaaagtacgtgccggtaagactcgcattgtcgacgtcctacctgttgaacacatcctctacaccaggatgatgattggcagattttgtgcacaaatgcactcaaacaacggaccccaaattggctcggcggtcggttgtaaccctgatgttgattggcaaagatttggcacacacttcgcccaatacagaaacgtgtgggatgtggactattcggccttcgatgctaaccactgcagtgacgccatgaacatcatgtttgaggaagtgtttcgcacagaattcgggttccacccaaacgctgagtggatcctgaagactctcgtgaacacggaacacgcctatgagaacaaacgcatcactgttgaaggcgggatgccatctggttgttccgcaacaagcatcatcaacacaattttgaacaacatctacgtgctctacgctttgcgtagacactatgagggagttgagctggacacttacaccatgatctcttacggagacgatatcgtggtggcaagtgattacgatttggactttgaggctctcaagccccacttcaaatcccttggtcaaaccatcactccagctgacaaaagcgacaaaggttttgttcttggtcactccattactgatgtcactttcctcaaaagacacttccacatggattatggaactgggttttacaaacctgtgatggcctcaaagacccttgaggctatcctctcctttgcacgccgtgggaccatacaggagaagttgatctccgtggcaggactcgctgttcactctggaccagacgagtaccggcgtctcttcgagccctttcaaggcctcttcgagattccaagctacagatcactttacctgcgttgggtgaacgccgtgtgcggcgacgcataatccctcagagactacattggcatactgtttctgaggcgcgcgacgccgtaggagtgaaaagcctgaaagggcttttcccgcttcctattccaaaaaaaaaaaaaaaaa

SEQ ID NO: 25 - DNA, 7597 bp, Artificial Sequence
  Fusion Nucleotide Sequence containing O1 Campos strain of FMD (complete genome)
ttgaaagggggcgctagggtctcacccctagcatgccaacgacagtccccgcgttgcactccacactcacgttgtgcgtgcgcggagctcgatggactatcgttcacccacctacagctggactcacggcaccgtgtggccacttggctggattgtgcggacgaacaccgcttgcgcttctcgcgtgaccggttagtactctcaccaccttccgcccacttggttgttagcgctgtcttgggcactcctgttgggggccgttcgacgctccgcgagtttccccgcacggcaactacggtgatggggccgtaccgcgcgggctgatcgcctggtgtgcttcggctgtcacccgaagcctacctttcaccccccccccccccccccccccccccccccccccccccccctaagttctaccgtcgttcccgacgtaaagggatgtaaccacaagcttactaccgcctttcccggcgttaaagggatgtaaccacaagacttaccttcacccggaagtaaaacggcaacttcacacagttttgcccgttttcatgagaaatgggacgtctgcgcacgaaacgcgccgtcgcttgaggaggacttgtacaaacacgatctaagcaggtttccccaactgacacaaaccgtgcaatttgaaactccgcctgggctttccaggtctagaggggtgacactttgtactgtgtttgactccacgttcgatccactggcgagtgttagtaacaacactgctgcttcgtagcggagcatgacggccgtgggacccccccccttggtaacaaggacccacggggccaaaagccacgtccgaatggacccgtcatgtgtgcaaacccagcacagtagctttgttgtgaaactcactttaaagtgacattgatactggtactcaagcactggtgacaggctaaggatgcccttcaggtaccccgaggtaacacgtgacactcgggatctgagaaggggaccggggcttctataaaagcgcccggtttaaaaagcttctatgtctgaataggtgaccggaggccggcacctttcttttaattacactggacttatgaacacaactgattgttttatcgctttggtacacgctatcagagagatcagagcatttttcctaccacgagccacaggaatgggggccggccaatccagtccggcgaccggctcgcagaaccaatctggcaacactggcagcataattaacaactactacatgcagcaataccagaactccatggacacacagcttggtgacaacgcaatcagtggaggctctaacgagggctccaccgacacaacctccacccacacaaccaacacccagaacaatgactggttctccaaacttgcaagctctgctttcagcggtcttttcggcgctcttctcgccgacaagaagacagaggagaccactctcctcgaagaccgcatcctcaccacccgtaacggccacaccacgtcgacaacccagtcaagcgttggagtcacatacgggtacgcaacagctgaggattttgtgagcggaccgaacacttccggtctcgagaccagagttgtgcaggcagaacggtttttcaaaacccacctcttcgactgggtcaccagtgactcattcggacgttgccacctcctggaactcccgaccgaccacaaaggtgtctacggcagcctgaccgactcgtatgcatatatgagaaacggctgggatgtcgaggtcaccgcggttggcaaccagttcaacggagggtgcctgctggtcgcaatggtaccagagcttcgttctatccaaaagagggaactgtaccagctcacacttttccctcaccagttcatcaacccacgcacgaacatgactgcgcacatcacagtgccctttgttggcgtcaaccgctacgaccagtacaaggttcacaagccttggacccttgtggttatggttgtagcccctctgaccgtcaacactgaaggtgcccctcagatcaaggtgtatgccaacattgccccaaccaacgtgcacgtcgcgggtgagtttccttccaaggagggaatattccccgtggcctgtagcgacggctatggtggcctggtgaccacggacccgaagacggctgaccccgtttatgggaaagtgttcaaccccccccgcaaccagttgccggggcgttttaccaacctccttgatgtggctgaggcatgcccgacgtttctgcacttcgagggtgacgtaccgtacgtgaccacgaaaacagactcggacagggtgcttgctcagtttgatatgtctttggcagcaaaacacatgtcaaacaccttcctcgcaggtcttgcgcagtactacacacagtacagtggcaccatcaacctgcacttcatgttcacaggacccactgacgcgaaggcgcgttacatgattgcctacgccccaccaggcatggagccgcccaagacacctgaggcggccgcgcactgcattcatgctgaatgggacactgggttgaactcaaagtttactttttccatcccctacctctcggccgccgattacgcgtacaccgcgtctgacgtggccgagaccacaaatgtgcagggatgggtctgcttgtttcaaattacacatggcaaggccgacggcgacgctctggtcgtactggctagtgctggtaaagactttgagctaaggctgccggtggacgcccgtgcggaaaccacttctgcgggcgagtcagcggatcctgtcaccgccactgttgaaaactacggtggcgaaacacagatccagaggcgccaacacacggacgtctcgttcatcatggacagatttgtgaaagtgacaccgcaaaaccaaattaacattttggacctcatgcagattccatcacacactttggtgggagcgctcctacgcgcgtccacttactacttctctgacttggagatagcagtaaaacacgagggagacctcacctgggttccaaatggagcgcctgaaaaggcgttggacaacaccaccaacccaactgcttaccacaaggcaccactcacccggcttgccctgccctacaccgcgccccaccgcgtgttggcaaccgtgtacaacggtgagtgcaggtacagcagaaatgctgtgcccaacgtgagaggtgaccttcaggtgttggctcaaaaggtggcacggacgctgcctacctccttcaactacggtgccatcaaagcgacccgggtcaccgagttgctttaccggatgaagagggccgaaacatactgtccaaggcccttgctggcaatccacccaactgaagccagacacaaacagaaaattgtggcaccggtgaaacagttctgaattttgaccttctcaagctagccggagacgttgagtccaaccctgggcccttcttcttctccgacgttaggtcaaacttttccaagctggtagacacaatcaaccagatgcaggaagacatgtccacaaagcacggacctgactttaaccggttggtgtccgcttttgaggagttggccactggagtgaaagccatcaggaccggtcttgacgaggccaagccctggtacaagcttatcaagctcctgagccgcctgtcgtgcatggccgctgtggcagcacggtcaaaggacccagtccttgtggccatcatgctggctgacaccggtctcgagattctggacagcaccttcgtcgtgaagaagatctccgactcgctctccagtctcttccacgtgccggcccccgtcttcagtttcggagccccgattctgttagccgggttggtcaaggtcgcctcgagtttcttccggtccacgcccgaagaccttgagagagcagagaaacagctcaaagcacgtgacatcaacgacattttcgccattctcaagaacggcgagtggctggtcaaattgatccttgccatccgcgactggatcaaggcatggatagcctcagaagaaaagtttgtcaccacgacagacttggtacctagcatccttgaaaaacagcaggacctcaacgacccaagcaagtacaaggaagccaaggagtggctcgacaacgcgcgccaagcgtgtttgaagagcgggaacgtccacattgccaacctgtgcaaagtggtcgccccggcacccagcaggtcgagacccgagcccgtggtcgtttgcctccgtggcaagtccggtcagggcaagagtttccttgcaaacgtgctcgcacaagcaatctctacccatttcactggcaggaccgattcagtttggtactgcccgcctgaccctgaccacttcgacggttacaaccaacagactgtcgttgtgatggacgatttgggccagaaccccgacggcaaagacttcaagtacttcgcccaaatggtttcaacaacggggttcatcccgcccatggcatcgcttgaggataaaggcaaacccttcaacagtaaggtcatcatagcaaccaccaacctgtactcgggcttcaccccgaggactatggtgtgccctgatgccctgaaccggaggtttcactttgacatcgacgtgagcgccaaggacgggtacaaaattaacaacaaattggacatcatcaaagcacttgaagatactcacaccaacccagtggcaatgtttcagtacgactgtgcccttctcaacggcatggctgttgaaatgaagagaatgcaacaagatatgttcaagcctcaaccaccccttcagaacgtgtaccaactggttcaagaggtgattgagcgggtggagctccacgagaaggtgtcgagccacccgattttcaaacagatctcaattccttcccaaaaatccgtgttgtacttcctcattgagaaaggacagcacgaggcagcaattgaattctttgagggcatggtgcacgactccatcaaggaggagctccggccgctcatccaacaaacctcatttgtgaaacgcgcttttaagcgcctgaaggaaaactttgagattgttgccctatgtctgaccctcctggccaacatagtgatcatgatccgcgaaactcgcaagagacagaagatggtggacgatgcagtgagtgagtacattgagagagcaaacatcaccaccgacgacaagactcttgatgaggcggaaaagaaccctctggaaaccagcggtgccagcaccgtcggcttcagagagagacctctcccaggccaaaaggcgcgtaatgacgagaactccgagcccgcccagcctgctgaagagcaaccacaagctgaaggaccctacgctggcccgatggagagaccagttaaagttaaagtgaaagcaaaagccccggtcgttaaggaaggaccttacgagggaccggtgaagaagcctgttgctttgaaagtgaaagctaagaacttgatcgtcactgagagtggtgccccaccgaccgacttgcaaaagttggtcatgggcaacaccaagcccgttgagctcatccttgacgggaagacggtagccatttgctgtgctactggagttttcggcactgcttacctcgtgcctcgtcatcttttcgcagaaaagtacgacaagatcatgttggacggcagagccatgacagatagtgactacagagtgtttgagtttgagattaaagtaaaaggacaggacatgctctcagacgctgcgctcatggtgctccaccgtgggaatcgcgtgagagacatcacgaaacactttcgtgacacagcaagaatgaagaaaggcacccccgtcgttggtgtgatcaacaacgccgatgtcgggagactgattttctctggtgaagcccttacctacaaggacattgtagtgtgcatggatggagacaccatgcctgggctctttgcctacaaagccgcaaccaaggctggttattgcggaggagccgtcctcgctaaggacggggctgacacgttcatcgttggcacccactccgctggaggcaatggcgttggatactgctcttgcgtttccaggtccatgcttctcaagatgaaggcacacgttgaccccgaaccacaccacgaggggttgattgttgacaccagagatgtggaagagcgcgttcacgtgatgcgcaaaaccaagcttgcacccaccgttgcgtacggtgtgttccgtcctgagttcgggcctgccgccttgtccaacaaggacccgcgcctgaacgacggtgttgtcctcgacgaagtcatcttctccaaacacaagggagacacaaagatgtctgaggaagacaaagcgctgttccgccgctgtgctgctgactacgcgtcacgcctgcacagcgtgttgggtacggcaaatgccccactgagcatctacgaggcaattaaaggcgttgatggactcgacgcaatggaaccagacaccgcacccggcctcccctgggcactccaggggaagcgccgtggcgcgctcatcgacttcgagaacggcactgttggacccgaagttgaggctgccttgaagctcatggagaaaagagaatacaagtttgcttgccaaaccttcctgaaggacgagattcgcccgatggagaaagtacgtgccggtaagactcgcattgtcgacgtcctacctgttgaacacatcctctacaccaggatgatgattggcagattttgtgcacaaatgcactcaaacaacggaccccaaattggctcggcggtcggttgtaaccctgatgttgattggcaaagatttggcacacacttcgcccaatacagaaacgtgtgggatgtggactattcggccttcgatgctaaccactgcagtgacgccatgaacatcatgtttgaggaagtgtttcgcacagaattcgggttccacccaaacgctgagtggatcctgaagactctcgtgaacacggaacacgcctatgagaacaaacgcatcactgttgaaggcgggatgccatctggttgttccgcaacaagcatcatcaacacaattttgaacaacatctacgtgctctacgctttgcgtagacactatgagggagttgagctggacacttacaccatgatctcttacggagacgatatcgtggtggcaagtgattacgatttggactttgaggctctcaagccccacttcaaatcccttggtcaaaccatcactccagctgacaaaagcgacaaaggttttgttcttggtcactccattactgatgtcactttcctcaaaagacacttccacatggattatggaactgggttttacaaacctgtgatggcctcaaagacccttgaggctatcctctcctttgcacgccgtgggaccatacaggagaagttgatctccgtggcaggactcgctgttcactctggaccagacgagtaccggcgtctcttcgagccctttcaaggcctcttcgagattccaagctacagatcactttacctgcgttgggtgaacgccgtgtgcggcgacgcataatccctcagagactacattggcatactgtttctgaggcgcgcgacgccgtaggagtgaaaagcctgaaagggcttttcccgcttcctattccaaaaaaaaaaaaaaaaaa

SEQ ID NO: 26 - DNA, 7586 bp, Artificial Sequence
  Fusion Nucleotide Sequence containing C3 Indaial strain of FMD (complete genome)
ttgaaagggggcgctagggtctcacccctagcatgccaacgacagtccccgcgttgcactccacactcacgttgtgcgtgcgcggagctcgatggactatcgttcacccacctacagctggactcacggcaccgtgtggccacttggctggattgtgcggacgaacaccgcttgcgcttctcgcgtgaccggttagtactctcaccaccttccgcccacttggttgttagcgctgtcttgggcactcctgttgggggccgttcgacgctccgcgagtttccccgcacggcaactacggtgatggggccgtaccgcgcgggctgatcgcctggtgtgcttcggctgtcacccgaagcctacctttcaccccccccccccccccccccccccccccccccccccccccctaagttctaccgtcgttcccgacgtaaagggatgtaaccacaagcttactaccgcctttcccggcgttaaagggatgtaaccacaagacttaccttcacccggaagtaaaacggcaacttcacacagttttgcccgttttcatgagaaatgggacgtctgcgcacgaaacgcgccgtcgcttgaggaggacttgtacaaacacgatctaagcaggtttccccaactgacacaaaccgtgcaatttgaaactccgcctgggctttccaggtctagaggggtgacactttgtactgtgtttgactccacgttcgatccactggcgagtgttagtaacaacactgctgcttcgtagcggagcatgacggccgtgggacccccccccttggtaacaaggacccacggggccaaaagccacgtccgaatggacccgtcatgtgtgcaaacccagcacagtagctttgttgtgaaactcactttaaagtgacattgatactggtactcaagcactggtgacaggctaaggatgcccttcaggtaccccgaggtaacacgtgacactcgggatctgagaaggggaccggggcttctataaaagcgcccggtttaaaaagcttctatgtctgaataggtgaccggaggccggcacctttcttttaattacactggacttatgaacacaactgattgttttatcgctttggtacacgctatcagagagatcagagcatttttcctaccacgagccacaggaatgggagccggacaatccagcccggcgactggctcgcagaaccaatctggcaacactggtagcataatcaacaactactacatgcaacagtaccaaaattccatggacacacagctgggtgacaatgctattagtggtggctccaacgagggctccacagatacaacttccacccacacaaccaacactcaaaacaacgactggttttccaaactcgccagttctgcctttagcggtcttttcggtgctcttcttgccgacaagaagaccgaggaaaccacactacttgaagaccgcatcctcaccacccgcaacggccacacgacgtcgacaactcagtcgagcgttggggtcacatacgggtacgcaacaactgaggatagcacgtcagggcccaacacatccggccttgagacacgtgttcaccaggcagaacggtttttcaagatgacactctttgaatgggttccctcccagagttttggacacatgcacaaggtcgttctgccctcagaaccgaaaggtgtctatgggggtctcgtcaagtcatacgcgtacatgcgcaatggctgggacgttgaggtgactgctgttggaaaccagttcaacggcggttgtctcctggtggcgctcgttcctgaaatgggtgacatcagtgacagagagaagtaccaactgactctctacccccaccaattcatcaacccacgcactaacatgacggcacacatcaccgtgccttacgtgggtgtcaacagatacgaccaatacaaccaacacaagccctggactcttgtcgtcatggtcgttgctccacttactgtgaacacatcaggtgcccagcagatcaaggtgtatgccaacatagccccaaccaacgttcacgttgctggtgaacttccctccaaggaggggatcttccccgttgcgtgtgccgacggctatggcaacatggtgacaactgacccgaagacagctgaccctgcctacgggaaagtctacaatccacccaggaccgccctgccgggccggttcacaaactacctggatgttgctgaggcttgccccactctcctgacgttcgagaacgtgccttacgtttcaacacggactgatggacaaaggctgttggccaagttcgacgtgtcattggcagcgaaacacatgtcaaacacttacttggctggcttggcccagtactacacacagtacgctgggacaatcaacctgcacttcatgttcactgggccaaccgacgcgaaagctcggtacatggtggcatacgtgccccctggcatggaagcaccagacaacccagaggaggctgcccactgcatacacgcagagtgggacactggtttgaactctaagttcacattttcaatcccgtacatctcggccgctgactacgcatacaccgcgtccagcgaggctgaaacaacaagcgtacagggatgggtttgtgtgtaccagatcactcacggcaaggcagacgctgacgcgctcgtcgtctccgcttcggcggggaaagactttgagctccggctacctgtggacgctagacagcaaactacgaccactggcgaatctgccgaccccgtcaccactaccgttgagaactacggaggagaaacacaaactcaacgtcgccaccacactgacgttgccttcgttcttgaccggtttgtgaaggtccaggtgtcgggcaaccaacacacactggacgttatgcaggtacacaaggacagtattgtgggtgcactcctacgcgcagccacatactacttctctgacttggaaatagcagtgactcacactgggaagctcacatgggtgcccaacggcgccccagtttctgcacttgacaacacaaccaaccccactgcctaccacaaggggccgctgactcggctggctctcccatacaccgcaccacaccgcgtgctggccacggcgtacaccggtacaacggcctacactaccggtgtacgcaggggagacctagcccacttggcggcggcgcacgctcggcacctgccgacgtcgttcaactttggtgcagttaaagcagagacaatcacagagctgcttgtgcgcatgaagcgtgctgaactctactgccccagaccggtccttccggtccaaccagcgggcgataggcacaaacaaccgctcattgcgccagcgaaacagcttctgaattttgacctgcttaagctagccggagacgttgagtccaaccctgggcccttcttcttctccgacgttaggtcaaacttttccaagctggtagacacaatcaaccagatgcaggaagacatgtccacaaagcacggacctgactttaaccggttggtgtccgcttttgaggagttggccactggagtgaaagccatcaggaccggtcttgacgaggccaagccctggtacaagcttatcaagctcctgagccgcctgtcgtgcatggccgctgtggcagcacggtcaaaggacccagtccttgtggccatcatgctggctgacaccggtctcgagattctggacagcaccttcgtcgtgaagaagatctccgactcgctctccagtctcttccacgtgccggcccccgtcttcagtttcggagccccgattctgttagccgggttggtcaaggtcgcctcgagtttcttccggtccacgcccgaagaccttgagagagcagagaaacagctcaaagcacgtgacatcaacgacattttcgccattctcaagaacggcgagtggctggtcaaattgatccttgccatccgcgactggatcaaggcatggatagcctcagaagaaaagtttgtcaccacgacagacttggtacctagcatccttgaaaaacagcaggacctcaacgacccaagcaagtacaaggaagccaaggagtggctcgacaacgcgcgccaagcgtgtttgaagagcgggaacgtccacattgccaacctgtgcaaagtggtcgccccggcacccagcaggtcgagacccgagcccgtggtcgtttgcctccgtggcaagtccggtcagggcaagagtttccttgcaaacgtgctcgcacaagcaatctctacccatttcactggcaggaccgattcagtttggtactgcccgcctgaccctgaccacttcgacggttacaaccaacagactgtcgttgtgatggacgatttgggccagaaccccgacggcaaagacttcaagtacttcgcccaaatggtttcaacaacggggttcatcccgcccatggcatcgcttgaggataaaggcaaacccttcaacagtaaggtcatcatagcaaccaccaacctgtactcgggcttcaccccgaggactatggtgtgccctgatgccctgaaccggaggtttcactttgacatcgacgtgagcgccaaggacgggtacaaaattaacaacaaattggacatcatcaaagcacttgaagatactcacaccaacccagtggcaatgtttcagtacgactgtgcccttctcaacggcatggctgttgaaatgaagagaatgcaacaagatatgttcaagcctcaaccaccccttcagaacgtgtaccaactggttcaagaggtgattgagcgggtggagctccacgagaaggtgtcgagccacccgattttcaaacagatctcaattccttcccaaaaatccgtgttgtacttcctcattgagaaaggacagcacgaggcagcaattgaattctttgagggcatggtgcacgactccatcaaggaggagctccggccgctcatccaacaaacctcatttgtgaaacgcgcttttaagcgcctgaaggaaaactttgagattgttgccctatgtctgaccctcctggccaacatagtgatcatgatccgcgaaactcgcaagagacagaagatggtggacgatgcagtgagtgagtacattgagagagcaaacatcaccaccgacgacaagactcttgatgaggcggaaaagaaccctctggaaaccagcggtgccagcaccgtcggcttcagagagagacctctcccaggccaaaaggcgcgtaatgacgagaactccgagcccgcccagcctgctgaagagcaaccacaagctgaaggaccctacgctggcccgatggagagaccagttaaagttaaagtgaaagcaaaagccccggtcgttaaggaaggaccttacgagggaccggtgaagaagcctgttgctttgaaagtgaaagctaagaacttgatcgtcactgagagtggtgccccaccgaccgacttgcaaaagttggtcatgggcaacaccaagcccgttgagctcatccttgacgggaagacggtagccatttgctgtgctactggagttttcggcactgcttacctcgtgcctcgtcatcttttcgcagaaaagtacgacaagatcatgttggacggcagagccatgacagatagtgactacagagtgtttgagtttgagattaaagtaaaaggacaggacatgctctcagacgctgcgctcatggtgctccaccgtgggaatcgcgtgagagacatcacgaaacactttcgtgacacagcaagaatgaagaaaggcacccccgtcgttggtgtgatcaacaacgccgatgtcgggagactgattttctctggtgaagcccttacctacaaggacattgtagtgtgcatggatggagacaccatgcctgggctctttgcctacaaagccgcaaccaaggctggttattgcggaggagccgtcctcgctaaggacggggctgacacgttcatcgttggcacccactccgctggaggcaatggcgttggatactgctcttgcgtttccaggtccatgcttctcaagatgaaggcacacgttgaccccgaaccacaccacgaggggttgattgttgacaccagagatgtggaagagcgcgttcacgtgatgcgcaaaaccaagcttgcacccaccgttgcgtacggtgtgttccgtcctgagttcgggcctgccgccttgtccaacaaggacccgcgcctgaacgacggtgttgtcctcgacgaagtcatcttctccaaacacaagggagacacaaagatgtctgaggaagacaaagcgctgttccgccgctgtgctgctgactacgcgtcacgcctgcacagcgtgttgggtacggcaaatgccccactgagcatctacgaggcaattaaaggcgttgatggactcgacgcaatggaaccagacaccgcacccggcctcccctgggcactccaggggaagcgccgtggcgcgctcatcgacttcgagaacggcactgttggacccgaagttgaggctgccttgaagctcatggagaaaagagaatacaagtttgcttgccaaaccttcctgaaggacgagattcgcccgatggagaaagtacgtgccggtaagactcgcattgtcgacgtcctacctgttgaacacatcctctacaccaggatgatgattggcagattttgtgcacaaatgcactcaaacaacggaccccaaattggctcggcggtcggttgtaaccctgatgttgattggcaaagatttggcacacacttcgcccaatacagaaacgtgtgggatgtggactattcggccttcgatgctaaccactgcagtgacgccatgaacatcatgtttgaggaagtgtttcgcacagaattcgggttccacccaaacgctgagtggatcctgaagactctcgtgaacacggaacacgcctatgagaacaaacgcatcactgttgaaggcgggatgccatctggttgttccgcaacaagcatcatcaacacaattttgaacaacatctacgtgctctacgctttgcgtagacactatgagggagttgagctggacacttacaccatgatctcttacggagacgatatcgtggtggcaagtgattacgatttggactttgaggctctcaagccccacttcaaatcccttggtcaaaccatcactccagctgacaaaagcgacaaaggttttgttcttggtcactccattactgatgtcactttcctcaaaagacacttccacatggattatggaactgggttttacaaacctgtgatggcctcaaagacccttgaggctatcctctcctttgcacgccgtgggaccatacaggagaagttgatctccgtggcaggactcgctgttcactctggaccagacgagtaccggcgtctcttcgagccctttcaaggcctcttcgagattccaagctacagatcactttacctgcgttgggtgaacgccgtgtgcggcgacgcataatccctcagagactacattggcatactgtttctgaggcgcgcgacgccgtaggagtgaaaagcctgaaagggcttttcccgcttcctattccaaaaaaaaaaaaaaaaaa

SEQ ID NO: 27 - DNA, 2076 bp, Artificial Sequence
  Fusion Nucleotide Sequence containing capsid and 2A partial sequence of C3 Indaial strain of FMD
ggggccggccaatccagcccagctactggctcgcagaaccaatctggtaacacaggtagcataatcaacaactactacatgcaacagtaccaaaactccatggacacacagcttggtgacaatgccatcagtggaggctctaacgagggctccacggacacaacttcaactcacacaaccaacacccaaaacaatgactggttttcaagactcgccggttcggccttctccggtttgtttggggccttgcttgccgacaagaagacggaggagacgacactccttgaggaccgcattctcaccactcgcaatgggcacaccacctccacgacccagtccagcgtaggcgttacatacgggtactccacaacagaggaccacgttgctggacccaacacatcaggtttggagacacgagtggtacaggcagagagattctacaaaaagtttttgtttgattggacaacggacaagccttttggacacctgcacaaactggagttgcccaccgaccaccacggtgttttcggacacttggtggactcatacgcctacatgaggaacggttgggacgttgaggtgtctgctgttggcaaccagttcaacggcggatgcctcctagtggccatggtacccgaatggaaagagtttgaaacgcgggagaagtaccagctcacgcttttcccgcaccagttcattagccccagaaccaacatgaccgcccacatcacggttccttaccttggtgtgaatagatatgatcagtacaaaaaacacaaaccctggacactggttgtcatggtcgtgtccccgctcacggtcaacgccacgagcgcggcacagatcaaggtctatgccaacatcgctccgacctacgttcatgtggccggcgagctcccctcgaaagaggggatcttccctgtcgcgtgcgcggacggttacggaggactggtgacaacggacccgaaaacagctgaccccgcctacggcaaggtgtacaatccgccccggactaactaccccgggcgtttcactaacttgttggacgtggctgaggcatgtcccacctttctgtgttttgacgacgggaaaccgtacgttaccacacagacaggtgagtctcgtcttctggccaagttcgacctttcccttgccgcgaagcacatgtctaacacatacttggcaggaattgcccagtactacacacagtactcaggcaccatcaatttgcatttcatgttcacaggttcaactgattcaaaagcccgctacatggtggcttacatcccgcctggggtggaaacaccaccggacacacctgagagggcagcccactgcatccatgctgagtgggacacagggctgaattccaaattcacattctcaatcccgtacgtgtctgccgcggattacgcctacacggcgtctgatgaggcagagacaacaaacgtacagggatgggtctgcgtttaccagatcacacacgggaaggctgacaacgacactctggtcgtgtcggttagcgccggcaaggacttcgagttgcgcctccccattgacccccgaccgcagaccaccgctactggggaatcagcagaccctgtcaccaccactgtagagaactacggcggtgagacacaagttcagagacgccaccacaccgacgttggcttcatcatggacagatttgtgaaaataaacagcccaaaatccacccatgttattgacctcatgcaaacccaccaacacggtctagtgggtgcgctgctgcgtgcggcgacctactacttctcagatctggaaattgttgtgcggcatgacggcaacctaacttgggtgcccaatggtgctcccgtgtcagccttgtccaacaccagcaaccccaccgcctacaacaaggcaccgttcacgagacttgccctcccctacaccgcgccacaccgcgtgttggcgactgtgtacaacgggacgagcaagtacactgtgagtgggtcaagcagacgaggcgacttgggttccctcgcggcacgagtcgtgaaggcacttcctgcttctttcaactacggtgcaatcaag

SEQ ID NO: 28 - DNA, 23 bp, Artificial Sequence
  Primer
gacaaaggttttgttcttggtca

SEQ ID NO: 29 - DNA, 18 bp, Artificial Sequence
  Primer
tgcgagtcctgccacgga

SEQ ID NO: 30 - DNA, 20 bp, Artificial Sequence
  Probe
tcctttgcacgccgtgggac